European Patent Specification EP 3 911 346 B1, published May 22, 2024. Title: Oral cavity treatments. Applicant: Rahimi, Maryam. The sequence listing filed with the application follows.

SEQUENCE LISTING (1 sequence)

SEQ ID NO: 1 - DNA, 12 bp, Allium cepa
ctcggttatggg